European Patent Specification EP 3 647 398 B1, published May 15, 2024. Title: Cleaning compositions containing dispersins V. Applicant: Henkel AG & Co. KGaA. The sequence listing filed with the application follows.

SEQUENCE LISTING (12 sequences)

SEQ ID NO: 1 - DNA, 1053 bp, Staphylococcus cohnii
  CDS (1)..(1050)
  sig_peptide (1)..(81)
  mat_peptide (82)..(1050)
gtggtctacattaaaattattttctcaacttcaattttactttcatatctttttttattcaactctttttctgtccatgctcaagattttcaaaagggaatcaatgttgatatagctagaaaagattattccttgaaatcactcaaaaagattgttgatacaattcatgagaataatggggattacttacaacttcatttttctgataatgaaaactatgcaattgaatctcaattttttaaacacgaaaatatagcttcacaaaattatttaagtcaacaagagttaaagaaccttattcattatagtaataagttaaatataatggttgttccagaatttgatttaccttctcattcaaaagcttggttattgttattaaaaaatgaaaattcaaacttacacgaaaatatcgtaagcgattatagcgatgaaacaattgattttttttctaatcaaaaagcattagagattagcaaaaggcaaatcaaagaaattttaaatctctttcatcaaccaaattttcaaaaagaacaaagaatagtattgggcggtgatgaggttcctggtggaaaatcataccaaaatgacttcattaattttatgaatgaaattggtgaatatgcttatcaaaatggatatgaaccacaaatatggaatgattctattactaaaaatggtttgaaattattaaaaaattacttttcagtaattttttggaaacaaagtaataatgaaaataatgaaccagggatcactgtcgaagattttttagactataattttaaagtttacaattataatttttattcactatattttttaccttctaaaaactatagcccaactgatatagaagaacaaactagctatatcagttgggcatataatcacaatagtttttactatttaaagaatccatattatgaagtagattctttaaatatccaaggttctgctttaagcttttggggcgagcatgctacaggcatgagagaggaagaagttctcaaccaagaactaccacttatacgcacatatttaaataaataa

SEQ ID NO: 2 - protein, 350 aa, Staphylococcus cohnii
VVYIKIIFSTSILLSYLFLFNSFSVHAQDFQKGINVDIARKDYSLKSLKKIVDTIHENNGDYLQLHFSDNENYAIESQFFKHENIASQNYLSQQELKNLIHYSNKLNIMVVPEFDLPSHSKAWLLLLKNENSNLHENIVSDYSDETIDFFSNQKALEISKRQIKEILNLFHQPNFQKEQRIVLGGDEVPGGKSYQNDFINFMNEIGEYAYQNGYEPQIWNDSITKNGLKLLKNYFSVIFWKQSNNENNEPGITVEDFLDYNFKVYNYNFYSLYFLPSKNYSPTDIEEQTSYISWAYNHNSFYYLKNPYYEVDSLNIQGSALSFWGEHATGMREEEVLNQELPLIRTYLNK

SEQ ID NO: 3 - protein, 323 aa, Staphylococcus cohnii
QDFQKGINVDIARKDYSLKSLKKIVDTIHENNGDYLQLHFSDNENYAIESQFFKHENIASQNYLSQQELKNLIHYSNKLNIMVVPEFDLPSHSKAWLLLLKNENSNLHENIVSDYSDETIDFFSNQKALEISKRQIKEILNLFHQPNFQKEQRIVLGGDEVPGGKSYQNDFINFMNEIGEYAYQNGYEPQIWNDSITKNGLKLLKNYFSVIFWKQSNNENNEPGITVEDFLDYNFKVYNYNFYSLYFLPSKNYSPTDIEEQTSYISWAYNHNSFYYLKNPYYEVDSLNIQGSALSFWGEHATGMREEEVLNQELPLIRTYLNK

SEQ ID NO: 4 - DNA, 1038 bp, Staphylococcus fleurettii
  CDS (1)..(1035)
  sig_peptide (1)..(72)
  mat_peptide (73)..(1035)
atgaaatttatttttgcacttgttataacttttttatttagcactgctttttcatttaaagatgtaagtgcagaaagtattcaagaaggtgtttcggtagacattgctagaaaagaatactcattagagtccttaaaacaaatagtcgatactattcatgaaaataatggacaatatcttcaattgcatttttctgatgatgaaaattatgcaatcgagtcagattatttctcgcatcaaggtattccaaatgaaaattatttaacaaaagcagaaataaaatcacttatagcatacagcaatgagttgaatgtaatggtagttccagatattgattttccttcccattcaaaagctcttttatcattgataaagaatgaggataaagatttgtataatcaaattattagtgactatagtgataatacgtttgattttttctcaaatgataaagctttagctataagtaagcgacacataggtgaaataacaacattatttaatcaaccaaaatataatggccagcaaagaatagtattaggtggagatgaagtgccaggcgggggtgcttaccaaagtgattttataagttatatgaataacattggaagttacgctgcagggcaaggttatgagcctcaaatgtggaacgatatgatttcgcatgaagggattaagtctttaaatgatacgttctcaattttatattggaaacaaaatgaaaacagtaaatcagatttaactgtagaagatttcgcggaatatgatttcaaaatatataattataacttttattcattatactttttaccatcgaatcaatttactaatgcagatatcgaagaacaagctgattacataagttgggcatatgcatataataagtttttctacactaatgaaccttatcaagaagtagacagtgacaacgtgaaaggatcagccttatcattttggggagaagatgcattgaatatgtcacaaacagaattgattaaccaagaaataccgttaataaaagcttatttcagttcgtga

SEQ ID NO: 5 - protein, 345 aa, Staphylococcus fleurettii
MKFIFALVITFLFSTAFSFKDVSAESIQEGVSVDIARKEYSLESLKQIVDTIHENNGQYLQLHFSDDENYAIESDYFSHQGIPNENYLTKAEIKSLIAYSNELNVMVVPDIDFPSHSKALLSLIKNEDKDLYNQIISDYSDNTFDFFSNDKALAISKRHIGEITTLFNQPKYNGQQRIVLGGDEVPGGGAYQSDFISYMNNIGSYAAGQGYEPQMWNDMISHEGIKSLNDTFSILYWKQNENSKSDLTVEDFAEYDFKIYNYNFYSLYFLPSNQFTNADIEEQADYISWAYAYNKFFYTNEPYQEVDSDNVKGSALSFWGEDALNMSQTELINQEIPLIKAYFSS

SEQ ID NO: 6 - protein, 321 aa, Staphylococcus fleurettii
ESIQEGVSVDIARKEYSLESLKQIVDTIHENNGQYLQLHFSDDENYAIESDYFSHQGIPNENYLTKAEIKSLIAYSNELNVMVVPDIDFPSHSKALLSLIKNEDKDLYNQIISDYSDNTFDFFSNDKALAISKRHIGEITTLFNQPKYNGQQRIVLGGDEVPGGGAYQSDFISYMNNIGSYAAGQGYEPQMWNDMISHEGIKSLNDTFSILYWKQNENSKSDLTVEDFAEYDFKIYNYNFYSLYFLPSNQFTNADIEEQADYISWAYAYNKFFYTNEPYQEVDSDNVKGSALSFWGEDALNMSQTELINQEIPLIKAYFSS

SEQ ID NO: 7 - protein, 27 aa, artificial
  signal peptide
MKKPLGKIVASTALLISVAFSSSIASA

SEQ ID NO: 8 - protein, 8 aa, artificial
  His-tag
HHHHHHPR

SEQ ID NO: 9 - protein, 4 aa, artificial
  motif
  Misc (2)..(2): Xaa = any of the 20 natural amino acids
GXDE

SEQ ID NO: 10 - protein, 7 aa, artificial
  motif
  Misc (1)..(1): Xaa = E (Glu) or Q (Gln)
  Misc (2)..(2): Xaa = N (Asn) or R (Arg) or S (Ser) or H (His) or A (Ala)
  Misc (3)..(3): Xaa = Y (Tyr) or V (Val) or F (Phe) or L(Leu)
  Misc (4)..(4): Xaa = A (Ala) or G (Gly) or S (Ser) or T (Thr) or C (Cys)
  Misc (5)..(5): Xaa = I (Ile) or V (Val) or L (Leu) or F (Phe)
  Misc (6)..(6): Xaa = E (Glu) or A (Ala) or Q (Gln) or Y (Tyr) or N (Asn)
  Misc (7)..(7): Xaa = S (Ser) or N (Asn)
XXXXXXX

SEQ ID NO: 11 - protein, 8 aa, artificial
  motif
  Misc (1)..(1): Xaa = V(Val) or I (Ile) or M (Met) or S (Ser)
  Misc (2)..(2): Xaa = L (Leu) or I (Ile) or V (Val)
  Misc (4)..(4): Xaa = G(Gly) or A (Ala) or V (Val)
  Misc (7)..(7): Xaa = V (Val) or I (Ile)
  Misc (8)..(8): Xaa = P (Pro) or S(Ser) or A(Ala)
XXGXDEXX

SEQ ID NO: 12 - protein, 5 aa, artificial
  motif
  Misc (2)..(2): Xaa = I (Ile) or V (Val)
  Misc (5)..(5): Xaa = T (Tyr) or K (Lys)
DXARX